European Patent Application EP 4 115 736 A1, published January 11, 2023. Title: BVP10 PROTEIN FOR CONTROLLING TETRANYCHID MITES AND USE THEREOF. Applicant: Hubei Biopesticide Engineering Research Center. The sequence listing filed with the application follows.

SEQUENCE LISTING (2 sequences)

SEQ ID NO: 1 - DNA, 270 bp, Artificial Sequence
atgttaaaaagtaaaattaaaaaaatagccggtgcggctgtaattgctggagcattattggtttctgtgtcgccagcaaaagcagaaactcttccgggattgatctgggtcatggacaaatatactgacgcttttaaattcgacatgtttattaaaaacggaaatgaaaaatgggtttatgtttacacaagattatccgatggcaaagttgatgtggaagaagtaaagtgtgaaacaatttataaagatcgatgctatgtaaagcagtaa

SEQ ID NO: 2 - protein, 89 aa, Artificial Sequence
MLKSKIKKIAGAAVIAGALLVSVSPAKAETLPGLIWVMDKYTDAFKFDMFIKNGNEKWVYVYTRLSDGKVDVEEVKCETIYKDRCYVKQ